European Patent Application EP 4 810 516 A1, published September 23, 2026. Title: TRGV9 BINDING PROTEINS AND MEDICAL USE THEREOF. Applicant: SHANGHAI SHENGDI PHARMACEUTICAL CO., LTD. Application WO. The sequence listing filed with the application follows.

SEQUENCE LISTING (73 sequences)

SEQ ID NO: 1 - protein, 298 aa, synthetic construct
  source 1..298: note = Recombinant human gamma 9 chain
AGHLEQPQISSTKTLSKTARLECVVSGITISATSVYWYRERPGEVIQFLVSISYDGTVRKESGIPSGKFEVDRIPETSTSTLTIHNVEKQDIATYYCALWEAQQELGKKIKVFGPGTKLIITDKQLDADVSPKPTIFLPSIAETKLQKAGTYLCLLEKFFPDVIKIHWEEKKSNTILGSCEGNTMKTNDTYMKFSWLTVPEKSLDKEHRCIVRHENNKNGVDQEIIFPPIKTDVITMDPKDNGSGLEVLFQGPGSGAQLEKELQALEKENAQLEWELQALEKELAQKGSGDYKDDDDK

SEQ ID NO: 2 - protein, 285 aa, synthetic construct
  source 1..285: note = Recombinant human delta 2 chain
AIELVPEHQTVPVSIGVPATLRCSMKGEAIGNYYINWYRKTQGNTMTFIYREKDIYGPGFKDNFQGDIDIAKNLAVLKILAPSERDEGSYYCACDTLGMGGEYTDKLIFGKGTRVTVEPRSQPHTKPSVFVMKNGTNVACLVKEFYPKDIRINLVSSKKITEFDPAICISPSGKYNAVKLGKYEDSNSVTCSVQHDNKTVHSTDFEVKTDSTDHVKPKETENTKQPSKSGSGLEVLFQGPGSGAQLKKKLQALKKKNAQLKWKLQALKKKLAQKGSGHHHHHHHH

SEQ ID NO: 3 - protein, 297 aa, synthetic construct
  source 1..297: note = Recombinant monkey gamma 9 chain
AGHLEQPQISSTKMLSKTARLECVVSGVTISETSIYWYRERPGEVIQFLVCIFYDGTVKKESSIPSGKFEVDRIPKTSTSTLTIHNVEKQDIATYYCALWEVQQFGRKVKLFGPGTKLIITDKHLDADVSPKPTIFLPSIAETNLHKAGTYLCLLENFFPDVIKIHWQEKKSNTILGSCEGNTVKTNDTYMKFSWLTVPEKSLDKEHRCIVRHENNKNGVDQEIIFPPIKTDVTTMDPKDNGSGLEVLFQGPGSGAQLEKELQALEKENAQLEWELQALEKELAQKGSGDYKDDDDK

SEQ ID NO: 4 - protein, 285 aa, synthetic construct
  source 1..285: note = Recombinant monkey delta 2 chain
AVELVPEHQTVIVSVGDPATLKCSMKGEAISNYYINWYRKTQGNTMTFIYREKGIYGPGFKDNFQGDIDTEENQAVLKILAPSERDEGSYYCASDILSWVDSYTDKLIFGKGTRVTVEPKRQPHTKPSVFVMKNGTNVACLVKDFYGKDIRINLESSKKITEFDPAICVSPSGKYNAVKLGQYADSNSVTCSVQHNKEVVYSTDFEVKTNSTDHLKPTETENTKQPSKSGSGLEVLFQGPGSGAQLKKKLQALKKKNAQLKWKLQALKKKLAQKGSGHHHHHHHH

SEQ ID NO: 5 - protein, 125 aa, synthetic construct
  source 1..125: note = SDP01346 VH
QVQLVESGGGLVQAGGSLRLSCTVSGSTFSDFAMGWLRQAPGKEREFVAAISWTGGRTYYADSVKGRFAISRDNGENTVYLQMNSLKSEDTAIYYCAASRDCSGPGCRVHEYDYWGQGTQVTVSS

SEQ ID NO: 6 - protein, 5 aa, synthetic construct
  source 1..5: note = CDR
DFAMG

SEQ ID NO: 7 - protein, 17 aa, synthetic construct
  source 1..17: note = CDR
AISWTGGRTYYADSVKG

SEQ ID NO: 8 - protein, 16 aa, synthetic construct
  source 1..16: note = CDR
SRDCSGPGCRVHEYDY

SEQ ID NO: 9 - protein, 116 aa, synthetic construct
  source 1..116: note = SDP01315 VH
EVKLVESGGGLVKPGGSLKLSCAASGFTFSSYAMSWVRQTPEKRLEWVASISSGGSTYYPDSVKGRFTISRDNARNILYLQMSSLRSEDTAMYYCARDGYPPFDYWGQGTTLTVSS

SEQ ID NO: 10 - protein, 107 aa, synthetic construct
  source 1..107: note = SDP01315 VL
DIVMTQSQKFMSTSVGDRVSVTCKASQNVGTNVAWYQQKPGQSPKALIYSASYRYSGVPDRFTGSGSGTDFTLTISNVQSEDLAEYFCQQYNSFPLTFGSGTKLEIK

SEQ ID NO: 11 - protein, 5 aa, synthetic construct
  source 1..5: note = HCDR1
SYAMS

SEQ ID NO: 12 - protein, 16 aa, synthetic construct
  source 1..16: note = HCDR2
SISSGGSTYYPDSVKG

SEQ ID NO: 13 - protein, 8 aa, synthetic construct
  source 1..8: note = HCDR3
DGYPPFDY

SEQ ID NO: 14 - protein, 11 aa, synthetic construct
  source 1..11: note = LCDR1
KASQNVGTNVA

SEQ ID NO: 15 - protein, 7 aa, synthetic construct
  source 1..7: note = LCDR2
SASYRYS

SEQ ID NO: 16 - protein, 9 aa, synthetic construct
  source 1..9: note = LCDR3
QQYNSFPLT

SEQ ID NO: 17 - protein, 136 aa, synthetic construct
  source 1..136: note = SDP01346
QVQLVESGGGLVQAGGSLRLSCTVSGSTFSDFAMGWLRQAPGKEREFVAAISWTGGRTYYADSVKGRFAISRDNGENTVYLQMNSLKSEDTAIYYCAASRDCSGPGCRVHEYDYWGQGTQVTVSSGGGGSHHHHHH

SEQ ID NO: 18 - protein, 446 aa, synthetic construct
  source 1..446: note = SDP01315 HC
EVKLVESGGGLVKPGGSLKLSCAASGFTFSSYAMSWVRQTPEKRLEWVASISSGGSTYYPDSVKGRFTISRDNARNILYLQMSSLRSEDTAMYYCARDGYPPFDYWGQGTTLTVSSASTKGPSVFPLAPSSKSTSGGTAALGCLVKDYFPEPVTVSWNSGALTSGVHTFPAVLQSSGLYSLSSVVTVPSSSLGTQTYICNVNHKPSNTKVDKKVEPKSCDKTHTCPPCPAPEFEGGPSVFLFPPKPKDTLMISRTPEVTCVVVDVSHEDPEVKFNWYVDGVEVHNAKTKPREEQYNSTYRVVSVLTVLHQDWLNGKEYKCKVSNKALPAPIEKTISKAKGQPREPQVYTLPPSREEMTKNQVSLTCLVKGFYPSDIAVEWESNGQPENNYKTTPPVLDSDGSFFLYSKLTVDKSRWQQGNVFSCSVMHEALHNHYTQKSLSLSPGK

SEQ ID NO: 19 - protein, 214 aa, synthetic construct
  source 1..214: note = SDP01315 LC
DIVMTQSQKFMSTSVGDRVSVTCKASQNVGTNVAWYQQKPGQSPKALIYSASYRYSGVPDRFTGSGSGTDFTLTISNVQSEDLAEYFCQQYNSFPLTFGSGTKLEIKRTVAAPSVFIFPPSDEQLKSGTASVVCLLNNFYPREAKVQWKVDNALQSGNSQESVTEQDSKDSTYSLSSTLTLSKADYEKHKVYACEVTHQGLSSPVTKSFNRGEC

SEQ ID NO: 20 - protein, 285 aa, synthetic construct
  source 1..285: note = Recombinant human delta 1 chain
AQKVTQAQSSVSMPVRKAVTLNCLYETSWWSYYIFWYKQLPSKEMIFLIRQGSDEQNAKSGRYSVNFKKAAKSVALTISALQLEDSAKYFCALGVRAFLRDWGIRVLIFGKGTRVTVEPRSQPHTKPSVFVMKNGTNVACLVKEFYPKDIRINLVSSKKITEFDPAICISPSGKYNAVKLGKYEDSNSVTCSVQHDNKTVHSTDFEVKTDSTDHVKPKETENTKQPSKSGSGLEVLFQGPGSGAQLKKKLQALKKKNAQLKWKLQALKKKLAQKGSGHHHHHHHH

SEQ ID NO: 21 - protein, 313 aa, synthetic construct
  source 1..313: note = Recombinant human gamma 8 chain
ADLSSNLEGRTKSVTRPTGSSAVITCDLPVENAVYTHWYLHQEGKAPQRLLYYDSYNSRVVLESGISREKYHTYASTGKSLKFILENLIERDSGVYYCATWASSDWIKTFAKGTRLIVTSPDKQLDADVSPKPTIFLPSIAETKLQKAGTYLCLLEKFFPDIIKIHWQEKKSNTILGSCEGNTMKTNDTYMKFSWLTVPEESLDKEHRCIVRHENNKNGIDQEIIFPPIKTDVTTVDPKYNYSKDANDVITMDPKDNGSGLEVLFQGPGSGAQLEKELQALEKENAQLEWELQALEKELAQKGSGDYKDDDDK

SEQ ID NO: 22 - protein, 308 aa, synthetic construct
  source 1..308: note = Recombinant human Vgamma 9Cbeta chain
AGHLEQPQISSTKTLSKTARLECVVSGITISATSVYWYRERPGEVIQFLVSISYDGTVRKESGIPSGKFEVDRIPETSTSTLTIHNVEKQDIATYYCALWEVHELGKKIKVFGPGTKLIITEDLKNVFPPEVAVFEPSEAEISHTQKATLVCLATGFYPDHVELSWWVNGKEVHSGVCTDPQPLKEQPALNDSRYSLSSRLRVSATFWQNPRNHFRCQVQFYGLSENDEWTQDRAKPVTQIVSAEAWGRADSGSGLEVLFQGPGSGAQLEKELQALEKENAQLEWELQALEKELAQKGSGDYKDDDDK

SEQ ID NO: 23 - protein, 271 aa, synthetic construct
  source 1..271: note = Recombinant human Vdelta 2Calpha chain
AIELVPEHQTVPVSIGVPATLRCSMKGEAIGNYYINWYRKTQGNTMTFIYREKDIYGPGFKDNFQGDIDIAKNLAVLKILAPSERDEGSYYCACDPVQVTGGYKVDKLIFGKGTRVTVEPNIQNPDPAVYQLRDSKSSDKSVCLFTDFDSQTNVSQSKDSDVYITDKCVLDMRSMDFKSNSAVAWSNKSDFACANAFNNSIIPEDTFFPSPESSSGSGLEVLFQGPGSGAQLKKKLQALKKKNAQLKWKLQALKKKLAQKGSGHHHHHHHH

SEQ ID NO: 24 - protein, 286 aa, synthetic construct
  source 1..286: note = Recombinant human Vbeta 7Cgamma chain
GVSQTPSNKVTEKGKYVELRCDPISGHTALYWYRQSLGQGPEFLIYFQGTGAADDSGLPNDRFFAVRPEGSVSTLKIQRTERGDSAVYLCATSALGDTQYFGPGTRLTVLDKQLDADVSPKPTIFLPSIAETKLQKAGTYLCLLEKFFPDVIKIHWEEKKSNTILGSCEGNTMKTNDTYMKFSWLTVPEKSLDKEHRCIVRHENNKNGVDQEIIFPPIKTDVITMDPKDNGSGLEVLFQGPGSGAQLEKELQALEKENAQLEWELQALEKELAQKGSGDYKDDDDK

SEQ ID NO: 25 - protein, 276 aa, synthetic construct
  source 1..276: note = Recombinant human Valpha 13Cdelta chain
ENVEQHPSTLSVQEGDSAVIKCTYSDSASNYFPWYKQELGKRPQLIIDIRSNVGEKKDQRIAVTLNKTAKHFSLHITETQPEDSAVYFCAASSFGNEKLTFGTGTRLTIIPSQPHTKPSVFVMKNGTNVACLVKEFYPKDIRINLVSSKKITEFDPAICISPSGKYNAVKLGKYEDSNSVTCSVQHDNKTVHSTDFEVKTDSTDHVKPKETENTKQPSKSGSGLEVLFQGPGSGAQLKKKLQALKKKNAQLKWKLQALKKKLAQKGSGHHHHHHHH

SEQ ID NO: 26 - protein, 125 aa, synthetic construct
  source 1..125: note = SDP01346 VH1
EVQLVESGGGVVQPGGSLRLSCAASGSTFSDFAMGWLRQAPGKGREFVAAISWTGGRTYYADSVKGRFTISRDNSKNTVYLQMNSLRAEDTAVYYCAASRDCSGPGCRVHEYDYWGQGTLVTVSS

SEQ ID NO: 27 - protein, 125 aa, synthetic construct
  source 1..125: note = SDP01346 VH2
EVQLVESGGGVVQPGGSLRLSCAVSGSTFSDFAMGWLRQAPGKEREFVAAISWTGGRTYYADSVKGRFTISRDNSKNTVYLQMNSLRAEDTAVYYCAASRDCSGPGCRVHEYDYWGQGTLVTVSS

SEQ ID NO: 28 - protein, 125 aa, synthetic construct
  source 1..125: note = SDP01346 VH3
EVQLVESGGGVVQPGGSLRLSCAVSGSTFSDFAMGWLRQAPGKEREFVAAISWTGGRTYYADSVKGRFTISRDNGKNTVYLQMNSLKSEDTAVYYCAASRDCSGPGCRVHEYDYWGQGTLVTVSS

SEQ ID NO: 29 - protein, 125 aa, synthetic construct
  source 1..125: note = SDP01346 VH4
EVQLVESGGGLVQPGGSLRLSCSVSGSTFSDFAMGWLRQAPGKEREFVAAISWTGGRTYYADSVKGRFTISRDNSKNTVYLQMNSLRAEDTAVYYCAASRDCSGPGCRVHEYDYWGQGTLVTVSS

SEQ ID NO: 30 - protein, 116 aa, synthetic construct
  source 1..116: note = SDP01315 VH1
EVQLVESGGGLVKPGGSLRLSCAASGFTFSSYAMSWVRQAPGKRLEWVSSISSGGSTYYPDSVKGRFTISRDNAKNSLYLQMNSLRAEDTAVYYCARDGYPPFDYWGQGTTVTVSS

SEQ ID NO: 31 - protein, 116 aa, synthetic construct
  source 1..116: note = SDP01315 VH2
EVQLVESGGGLVKPGGSLRLSCAASGFTFSSYAMSWVRQAPGKRLEWVASISSGGSTYYPDSVKGRFTISRDNAKNSLYLQMNSLRAEDTAVYYCARDGYPPFDYWGQGTTVTVSS

SEQ ID NO: 32 - protein, 116 aa, synthetic construct
  source 1..116: note = SDP01315 VH3
EVQLVESGGGLVQPGGSLRLSCAASGFTFSSYAMSWVRQAPGKRLEWVASISSGGSTYYPDSVKGRFTISRDNAKNTLYLQMNSLRAEDTAVYYCARDGYPPFDYWGQGTLVTVSS

SEQ ID NO: 33 - protein, 107 aa, synthetic construct
  source 1..107: note = SDP01315 VL1
DIQMTQSPSSVSASVGDRVTITCKASQNVGTNVAWYQQKPGKAPKLLIYSASYRYSGVPSRFSGSGSGTDFTLTISSLQPEDFATYYCQQYNSFPLTFGQGTKLEIK

SEQ ID NO: 34 - protein, 107 aa, synthetic construct
  source 1..107: note = SDP01315 VL2
DIQMTQSPSSVSASVGDRVTITCKASQNVGTNVAWYQQKPGKAPKALIYSASYRYSGVPSRFSGSGSGTDFTLTISSLQPEDFATYYCQQYNSFPLTFGQGTKLEIK

SEQ ID NO: 35 - protein, 107 aa, synthetic construct
  source 1..107: note = SDP01315 VL3
DIQMTQSPSSVSASVGDRVTVTCKASQNVGTNVAWYQQKPGKSPKALIYSASYRYSGVPSRFSGSGSGTDFTLTISSLQPEDFATYFCQQYNSFPLTFGQGTKLEIK

SEQ ID NO: 36 - protein, 136 aa, synthetic construct
  source 1..136: note = SDP01378
EVQLVESGGGLVQPGGSLRLSCSVSGSTFSDFAMGWLRQAPGKEREFVAAISWTGGRTYYADSVKGRFTISRDNSKNTVYLQMNSLRAEDTAVYYCAASRDCSGPGCRVHEYDYWGQGTLVTVSSGGGGSHHHHHH

SEQ ID NO: 37 - protein, 446 aa, synthetic construct
  source 1..446: note = SDP01369 HC
EVQLVESGGGLVKPGGSLRLSCAASGFTFSSYAMSWVRQAPGKRLEWVASISSGGSTYYPDSVKGRFTISRDNAKNSLYLQMNSLRAEDTAVYYCARDGYPPFDYWGQGTTVTVSSASTKGPSVFPLAPSSKSTSGGTAALGCLVKDYFPEPVTVSWNSGALTSGVHTFPAVLQSSGLYSLSSVVTVPSSSLGTQTYICNVNHKPSNTKVDKKVEPKSCDKTHTCPPCPAPEFEGGPSVFLFPPKPKDTLMISRTPEVTCVVVDVSHEDPEVKFNWYVDGVEVHNAKTKPREEQYNSTYRVVSVLTVLHQDWLNGKEYKCKVSNKALPAPIEKTISKAKGQPREPQVYTLPPSREEMTKNQVSLTCLVKGFYPSDIAVEWESNGQPENNYKTTPPVLDSDGSFFLYSKLTVDKSRWQQGNVFSCSVMHEALHNHYTQKSLSLSPGK

SEQ ID NO: 38 - protein, 214 aa, synthetic construct
  source 1..214: note = SDP01369 LC
DIQMTQSPSSVSASVGDRVTITCKASQNVGTNVAWYQQKPGKAPKALIYSASYRYSGVPSRFSGSGSGTDFTLTISSLQPEDFATYYCQQYNSFPLTFGQGTKLEIKRTVAAPSVFIFPPSDEQLKSGTASVVCLLNNFYPREAKVQWKVDNALQSGNSQESVTEQDSKDSTYSLSSTLTLSKADYEKHKVYACEVTHQGLSSPVTKSFNRGEC

SEQ ID NO: 39 - protein, 115 aa, synthetic construct
  source 1..115: note = GPC3 VH
QVQLVQSGAEVKKPGASVKVSCKASGYTFTDYEMHWVRQAPGQGLEWMGALDPKTGDTAYSQKFKGRVTLTADKSTSTAYMELSSLTSEDTAVYYCTRFYSYTYWGQGTLVTVSS

SEQ ID NO: 40 - protein, 112 aa, synthetic construct
  source 1..112: note = GPC3 VL
DVVMTQSPLSLPVTPGEPASISCRSSQSLVHSNRNTYLHWYLQKPGQSPQLLIYKVSNRFSGVPDRFSGSGSGTDFTLKISRVEAEDVGVYYCSQNTHVPPTFGQGTKLEIK

SEQ ID NO: 41 - protein, 5 aa, synthetic construct
  source 1..5: note = HCDR1
DYEMH

SEQ ID NO: 42 - protein, 17 aa, synthetic construct
  source 1..17: note = HCDR2
ALDPKTGDTAYSQKFKG

SEQ ID NO: 43 - protein, 6 aa, synthetic construct
  source 1..6: note = HCDR3
FYSYTY

SEQ ID NO: 44 - protein, 16 aa, synthetic construct
  source 1..16: note = LCDR1
RSSQSLVHSNRNTYLH

SEQ ID NO: 45 - protein, 7 aa, synthetic construct
  source 1..7: note = LCDR2
KVSNRFS

SEQ ID NO: 46 - protein, 9 aa, synthetic construct
  source 1..9: note = LCDR3
SQNTHVPPT

SEQ ID NO: 47 - protein, 97 aa, synthetic construct
  source 1..97: note = Obscurin-O
SGAPRFLTRPKASVVSVGKDATLSCQIVGNPFPQVSWEKDKQPVTAGVRFRLAQDGDLYRLKILDLQLSDSGQYVCRARNAHGEAFACLGLQVDAEA

SEQ ID NO: 48 - protein, 98 aa, synthetic construct
  source 1..98: note = Titin-T
GIPPKIECLPIDISIDEGKVLTVASAFTGEPTPEVTWSTGGRKIHSQEQGRFHIENTDDSTTLTIKDVQKQDGGLYTLTLRNEFGSDSATVNIHIRSI

SEQ ID NO: 49 - protein, 103 aa, synthetic construct
  source 1..103: note = CH1
ASTKGPSVFPLAPSSKSTSGGTAALGCLVKDYFPEPVTVSWNSGALTSGVHTFPAVLQSSGLYSLSSVVTVPSSSLGTQTYICNVNHKPSNTKVDKKVEPKSC

SEQ ID NO: 50 - protein, 107 aa, synthetic construct [sequence omitted]

SEQ ID NO: 51 - protein, 227 aa, synthetic construct
  source 1..227: note = IgG1 Fc
DKTHTCPPCPAPELLGGPSVFLFPPKPKDTLMISRTPEVTCVVVDVSHEDPEVKFNWYVDGVEVHNAKTKPREEQYNSTYRVVSVLTVLHQDWLNGKEYKCKVSNKALPAPIEKTISKAKGQPREPQVYTLPPSREEMTKNQVSLTCLVKGFYPSDIAVEWESNGQPENNYKTTPPVLDSDGSFFLYSKLTVDKSRWQQGNVFSCSVMHEALHNHYTQKSLSLSPGK

SEQ ID NO: 52 - protein, 227 aa, synthetic construct
  source 1..227: note = IgG1 Fc1
DKTHTCPPCPAPEFEGGPSVFLFPPKPKDTLMISRTPEVTCVVVDVSHEDPEVKFNWYVDGVEVHNAKTKPREEQYNSTYRVVSVLTVLHQDWLNGKEYKCKVSNKALPAPIEKTISKAKGQPREPQVYTLPPCREEMTKNQVSLWCLVKGFYPSDIAVEWESNGQPENNYKTTPPVLDSDGSFFLYSKLTVDKSRWQQGNVFSCSVMHEALHNHYTQKSLSLSPGK

SEQ ID NO: 53 - protein, 227 aa, synthetic construct
  source 1..227: note = IgG1 Fc2
DKTHTCPPCPAPEFEGGPSVFLFPPKPKDTLMISRTPEVTCVVVDVSHEDPEVKFNWYVDGVEVHNAKTKPREEQYNSTYRVVSVLTVLHQDWLNGKEYKCKVSNKALPAPIEKTISKAKGQPREPQVCTLPPSREEMTKNQVSLSCAVKGFYPSDIAVEWESNGQPENNYKTTPPVLDSDGSFFLVSKLTVDKSRWQQGNVFSCSVMHEALHNHYTQKSLSLSPGK

SEQ ID NO: 54 - protein, 356 aa, synthetic construct
  source 1..356: note = SDP01716 H1
EVQLVESGGGLVQPGGSLRLSCSVSGSTFSDFAMGWLRQAPGKEREFVAAISWTGGRTYYADSVKGRFTISRDNSKNTVYLQMNSLRAEDTAVYYCAASRDCSGPGCRVHEYDYWGQGTLVTVSSAAASDKTHTCPPCPAPEFEGGPSVFLFPPKPKDTLMISRTPEVTCVVVDVSHEDPEVKFNWYVDGVEVHNAKTKPREEQYNSTYRVVSVLTVLHQDWLNGKEYKCKVSNKALPAPIEKTISKAKGQPREPQVYTLPPCREEMTKNQVSLWCLVKGFYPSDIAVEWESNGQPENNYKTTPPVLDSDGSFFLYSKLTVDKSRWQQGNVFSCSVMHEALHNHYTQKSLSLSPGK

SEQ ID NO: 55 - protein, 411 aa, synthetic construct
  source 1..411: note = SDP01716 H2
QVQLVQSGAEVKKPGASVKVSCKASGYTFTDYEMHWVRQAPGQGLEWMGALDPKTGDTAYSQKFKGRVTLTADKSTSTAYMELSSLTSEDTAVYYCTRFYSYTYWGQGTLVTVSSASTKGPSVFPLAPSSKSTSGGTAALGCLVKDYFPEPVTVSWNSGALTSGVHTFPAVLQSSGLYSLSSVVTVPSSSLGTQTYICNVNHKPSNTKVDKKVEPKSCDKTHTCPPCPAPEFEGGPSVFLFPPKPKDTLMISRTPEVTCVVVDVSHEDPEVKFNWYVDGVEVHNAKTKPREEQYNSTYRVVSVLTVLHQDWLNGKEYKCKVSNKALPAPIEKTISKAKGQPREPQVCTLPPSREEMTKNQVSLSCAVKGFYPSDIAVEWESNGQPENNYKTTPPVLDSDGSFFLVSKLTVD

SEQ ID NO: 56 - protein, 219 aa, synthetic construct
  source 1..219: note = SDP01716 L
DVVMTQSPLSLPVTPGEPASISCRSSQSLVHSNRNTYLHWYLQKPGQSPQLLIYKVSNRFSGVPDRFSGSGSGTDFTLKISRVEAEDVGVYYCSQNTHVPPTFGQGTKLEIKRTVAAPSVFIFPPSDEQLKSGTASVVCLLNNFYPREAKVQWKVDNALQSGNSQESVTEQDSKDSTYSLSSTLTLSKADYEKHKVYACEVTHQGLSSPVTKSFNRGEC

SEQ ID NO: 57 - protein, 445 aa, synthetic construct
  source 1..445: note = SDP01696 H1
EVQLVESGGGLVKPGGSLRLSCAASGFTFSSYAMSWVRQAPGKRLEWVASISSGGSTYYPDSVKGRFTISRDNAKNSLYLQMNSLRAEDTAVYYCARDGYPPFDYWGQGTTVTVSSGGGGSSGAPRFLTRPKASVVSVGKDATLSCQIVGNPFPQVSWEKDKQPVTAGVRFRLAQDGDLYRLKILDLQLSDSGQYVCRARNAHGEAFACLGLQVDAEADKTHTCPPCPAPEFEGGPSVFLFPPKPKDTLMISRTPEVTCVVVDVSHEDPEVKFNWYVDGVEVHNAKTKPREEQYNSTYRVVSVLTVLHQDWLNGKEYKCKVSNKALPAPIEKTISKAKGQPREPQVYTLPPCREEMTKNQVSLWCLVKGFYPSDIAVEWESNGQPENNYKTTPPVLDSDGSFFLYSKLTVDKSRWQQGNVFSCSVMHEALHNHYTQKSLSLSPGK

SEQ ID NO: 58 - protein, 210 aa, synthetic construct
  source 1..210: note = SDP01696 L1
DIQMTQSPSSVSASVGDRVTITCKASQNVGTNVAWYQQKPGKAPKALIYSASYRYSGVPSRFSGSGSGTDFTLTISSLQPEDFATYYCQQYNSFPLTFGQGTKLEIKGGGGSGIPPKIECLPIDISIDEGKVLTVASAFTGEPTPEVTWSTGGRKIHSQEQGRFHIENTDDSTTLTIKDVQKQDGGLYTLTLRNEFGSDSATVNIHIRSI

SEQ ID NO: 59 - protein, 445 aa, synthetic construct
  source 1..445: note = SDP01696 H2
QVQLVQSGAEVKKPGASVKVSCKASGYTFTDYEMHWVRQAPGQGLEWMGALDPKTGDTAYSQKFKGRVTLTADKSTSTAYMELSSLTSEDTAVYYCTRFYSYTYWGQGTLVTVSSASTKGPSVFPLAPSSKSTSGGTAALGCLVKDYFPEPVTVSWNSGALTSGVHTFPAVLQSSGLYSLSSVVTVPSSSLGTQTYICNVNHKPSNTKVDKKVEPKSCDKTHTCPPCPAPEFEGGPSVFLFPPKPKDTLMISRTPEVTCVVVDVSHEDPEVKFNWYVDGVEVHNAKTKPREEQYNSTYRVVSVLTVLHQDWLNGKEYKCKVSNKALPAPIEKTISKAKGQPREPQVCTLPPSREEMTKNQVSLSCAVKGFYPSDIAVEWESNGQPENNYKTTPPVLDSDGSFFLVSKLTVDKSRWQQGNVFSCSVMHEALHNHYTQKSLSLSPGK

SEQ ID NO: 60 - protein, 674 aa, synthetic construct
  source 1..674: note = SDP01704 H2
QVQLVQSGAEVKKPGASVKVSCKASGYTFTDYEMHWVRQAPGQGLEWMGALDPKTGDTAYSQKFKGRVTLTADKSTSTAYMELSSLTSEDTAVYYCTRFYSYTYWGQGTLVTVSSASTKGPSVFPLAPSSKSTSGGTAALGCLVKDYFPEPVTVSWNSGALTSGVHTFPAVLQSSGLYSLSSVVTVPSSSLGTQTYICNVNHKPSNTKVDKKVEPKSCDGGGGSGGGGSQVQLVQSGAEVKKPGASVKVSCKASGYTFTDYEMHWVRQAPGQGLEWMGALDPKTGDTAYSQKFKGRVTLTADKSTSTAYMELSSLTSEDTAVYYCTRFYSYTYWGQGTLVTVSSASTKGPSVFPLAPSSKSTSGGTAALGCLVKDYFPEPVTVSWNSGALTSGVHTFPAVLQSSGLYSLSSVVTVPSSSLGTQTYICNVNHKPSNTKVDKKVEPKSCDKTHTCPPCPAPEFEGGPSVFLFPPKPKDTLMISRTPEVTCVVVDVSHEDPEVKFNWYVDGVEVHNAKTKPREEQYNSTYRVVSVLTVLHQDWLNGKEYKCKVSNKALPAPIEKTISKAKGQPREPQVCTLPPSREEMTKNQVSLSCAVKGFYPSDIAVEWESNGQPENNYKTTPPVLDSDGSFFLVSKLTVDKSRWQQGNVFSCSVMHEALHNHYTQKSLSLSPGK

SEQ ID NO: 61 - protein, 219 aa, synthetic construct; identical to SEQ ID NO: 56
  source 1..219: note = SDP01704 L2

SEQ ID NO: 62 - protein, 5 aa, synthetic construct
  source 1..5: note = linker
GGNGT

SEQ ID NO: 63 - protein, 5 aa, synthetic construct
  source 1..5: note = linker
YGNGT

SEQ ID NO: 64 - protein, 5 aa, synthetic construct
  source 1..5: note = linker
EPKSS

SEQ ID NO: 65 - protein, 5 aa, synthetic construct
  source 1..5: note = linker
GGGGS

SEQ ID NO: 66 - protein, 10 aa, synthetic construct
  source 1..10: note = linker
GGGGSGGGGS

SEQ ID NO: 67 - protein, 15 aa, synthetic construct
  source 1..15: note = linker
GGGGSGGGGSGGGGS

SEQ ID NO: 68 - protein, 20 aa, synthetic construct
  source 1..20: note = linker
GGGGSGGGGSGGGGSGGGGS

SEQ ID NO: 69 - protein, 25 aa, synthetic construct
  source 1..25: note = linker
GGGGSGGGGSGGGGSGGGGSGGGGS

SEQ ID NO: 70 - protein, 4 aa, synthetic construct
  source 1..4: note = linker
ASGS

SEQ ID NO: 71 - protein, 4 aa, synthetic construct
  source 1..4: note = linker
AAAS

SEQ ID NO: 72 - protein, 11 aa, synthetic construct
  source 1..11: note = Sequence after VHH
GGGGSHHHHHH

SEQ ID NO: 73 - protein, 356 aa, synthetic construct
  source 1..356: note = SDP05576
EVQLVESGGGLVQPGGSLRLSCSVSGSTFSDFAMGWLRQAPGKEREFVAAISWTGGRTYYADSVKGRFTISRDNSKNTVYLQMNSLRAEDTAVYYCAASRDCSGPGCRVHEYDYWGQGTLVTVSSAAASDKTHTCPPCPAPELLGGPSVFLFPPKPKDTLMISRTPEVTCVVVDVSHEDPEVKFNWYVDGVEVHNAKTKPREEQYNSTYRVVSVLTVLHQDWLNGKEYKCKVSNKALPAPIEKTISKAKGQPREPQVYTLPPSREEMTKNQVSLTCLVKGFYPSDIAVEWESNGQPENNYKTTPPVLDSDGSFFLYSKLTVDKSRWQQGNVFSCSVMHEALHNHYTQKSLSLSPGK